European Patent Specification EP 3 845 240 B1, published November 6, 2024. Title: Novel proinsulin aspart and method for preparing insulin aspart. Applicant: Amphastar Nanjing Pharmaceuticals Inc. The sequence listing filed with the application follows.

SEQUENCE LISTING (21 sequences)

SEQ ID NO: 1 - protein, 63 aa, Artificial sequence
  The sequence is synthesized
MATHAVSVLKGDGPVQGIINFEQHESNGPVKVWGSIHGLTEGLHGFHVHEFGDNTAGSTSAGP

SEQ ID NO: 2 - protein, 63 aa, Artificial sequence
  The sequence is synthesized
MATKAVSVLKGDGPVQGIINFEQKESNGPVKVWGSIKGLTEGLHGFHVHEFGDNTAGSTSAGP

SEQ ID NO: 3 - protein, 1 aa, Artificial sequence
  The sequence is synthesized
R

SEQ ID NO: 4 - protein, 1 aa, Artificial sequence
  The sequence is synthesized
K

SEQ ID NO: 5 - protein, 21 aa, Native human insulin A chain
GIVEQCCTSICSLYQLENYCN

SEQ ID NO: 6 - protein, 30 aa, Native human insulin B chain
FVNQHLCGSHLVEALYLVCGERGFFYTPKT

SEQ ID NO: 7 - protein, 35 aa, Native human insulin C peptide
RREAEDLQVGQVELGGGPGAGSLQPLALEGSLQKR

SEQ ID NO: 8 - protein, 1 aa, Artificial sequence
  The sequence is synthesized
R

SEQ ID NO: 9 - protein, 1 aa, Artificial sequence
  The sequence is synthesized
K

SEQ ID NO: 10 - protein, 86 aa, Native human proinsulin
FVNQHLCGSHLVEALYLVCGERGFFYTPKTRREAEDLQVGQVELGGGPGAGSLQPLALEGSLQKRGIVEQCCTSICSLYQLENYCN

SEQ ID NO: 11 - protein, 53 aa, Artificial sequence
  The sequence is synthesized
FVNQHLCGSHLVEALYLVCGERGFFYTDKAAKGIVEQCCTSICSLYQLENYCN

SEQ ID NO: 12 - protein, 52 aa, Artificial sequence
  The sequence is synthesized
FVNQHLCGSHLVEALYLVCGERGFFYTDKTRGIVEQCCTSICSLYQLENYCN

SEQ ID NO: 13 - protein, 52 aa, Artificial sequence
  The sequence is synthesized
FVNQHLCGSHLVEALYLVCGERGFFYTDKTKGIVEQCCTSICSLYQLENYCN

SEQ ID NO: 14 - protein, 116 aa, Artificial sequence
  The sequence is synthesized
MATHAVSVLKGDGPVQGIINFEQHESNGPVKVWGSIHGLTEGLHGFHVHEFGDNTAGSTSAGPRFVNQHLCGSHLVEALYLVCGERGFFYTDKTRGIVEQCCTSICSLYQLENYCN

SEQ ID NO: 15 - protein, 116 aa, Artificial sequence
  The sequence is synthesized
MATHAVSVLKGDGPVQGIINFEQHESNGPVKVWGSIHGLTEGLHGFHVHEFGDNTAGSTSAGPKFVNQHLCGSHLVEALYLVCGERGFFYTDKTKGIVEQCCTSICSLYQLENYCN

SEQ ID NO: 16 - protein, 116 aa, Artificial sequence
  The sequence is synthesized
MATKAVSVLKGDGPVQGIINFEQKESNGPVKVWGSIKGLTEGLHGFHVHEFGDNTAGSTSAGPRFVNQHLCGSHLVEALYLVCGERGFFYTDKTRGIVEQCCTSICSLYQLENYCN

SEQ ID NO: 17 - protein, 116 aa, Artificial sequence
  The sequence is synthesized
MATKAVSVLKGDGPVQGIINFEQKESNGPVKVWGSIKGLTEGLHGFHVHEFGDNTAGSTSAGPKFVNQHLCGSHLVEALYLVCGERGFFYTDKTKGIVEQCCTSICSLYQLENYCN

SEQ ID NO: 18 - DNA, 351 bp, Artificial sequence
  The sequence is synthesized
atggcgacgcatgccgtgagcgtgctgaagggcgacggcccagtgcagggcatcatcaatttcgagcagcatgaaagtaatggaccagtgaaggtgtggggaagcattcatggactgactgaaggcctgcatggattccatgttcatgagtttggagataatacagctggctctaccagtgcaggtccgcggtttgtgaaccagcatctgtgcggcagccatctggtggaagcgctgtatctggtgtgcggcgaacgcggcttcttttataccgataaaacccgcggcattgtggaacagtgctgcaccagcatttgcagcctgtatcagctggaaaactattgcaactaa

SEQ ID NO: 19 - DNA, 351 bp, Artificial sequence
  The sequence is synthesized
atggcgacgcatgccgtgagcgtgctgaagggcgacggcccagtgcagggcatcatcaatttcgagcagcatgaaagtaatggaccagtgaaggtgtggggaagcattcatggactgactgaaggcctgcatggattccatgttcatgagtttggagataatacagctggctctaccagtgcaggtccgaaatttgtgaaccagcatctgtgcggcagccatctggtggaagcgctgtatctggtgtgcggcgaacgcggcttcttttataccgataaaacccgcggcattgtggaacagtgctgcaccagcatttgcagcctgtatcagctggaaaactattgcaactaa

SEQ ID NO: 20 - DNA, 351 bp, Artificial sequence
  The sequence is synthesized
atggcgacgaaagccgtgagcgtgctgaagggcgacggcccagtgcagggcatcatcaatttcgagcagaaagaaagtaatggaccagtgaaggtgtggggaagcattaaaggactgactgaaggcctgcatggattccatgttcatgagtttggagataatacagctggctctaccagtgcaggtccgcggtttgtgaatcagcatctgtgcggcagccatctggtggaagcgctgtatctggtgtgcggcgaacgcggcttcttttataccgataaaacccgcggcattgtggaacagtgctgcaccagcatttgcagcctgtatcagctggaaaattattgcaactaa

SEQ ID NO: 21 - DNA, 351 bp, Artificial sequence
  The sequence is synthesized
atggcgacgaaagccgtgagcgtgctgaagggcgacggcccagtgcagggcatcatcaatttcgagcagaaagaaagtaatggaccagtgaaggtgtggggaagcattaaaggactgactgaaggcctgcatggattccatgttcatgagtttggagataatacagctggctctaccagtgcaggtccgaaatttgtgaatcagcatctgtgcggcagccatctggtggaagcgctgtatctggtgtgcggcgaacgcggcttcttttataccgataaaacccgcggcattgtggaacagtgctgcaccagcatttgcagcctgtatcagctggaaaattattgcaactaa